European Patent Application EP 4 403 571 A1, published July 24, 2024. Title: HUMAN EPIDERMAL GROWTH FACTOR RECEPTOR BINDING MOLECULE AND USE THEREOF. Applicant: ZHEJIANG NANOMAB TECHNOLOGY CENTER CO. LTD. The sequence listing filed with the application follows.

SEQUENCE LISTING (87 sequences)

SEQ ID NO: 1 - protein, 8 aa, Artificial Sequence
  CDR1
  MUTAGEN (1)..(1): Xaa is G
  MUTAGEN (2)..(2): Xaa is S, F, G, L or R
  MUTAGEN (3)..(3): Xaa is G, T, V, P, A, S or I
  MUTAGEN (4)..(4): Xaa is F, L or D
  MUTAGEN (5)..(5): Xaa is T, S, E, D, L or I
  MUTAGEN (6)..(6): Xaa is I, D, S or T
  MUTAGEN (7)..(7): Xaa is Q, Y, H or F
  MUTAGEN (8)..(8): Xaa is A or T
XXXXXXXX

SEQ ID NO: 2 - protein, 8 aa, Artificial Sequence
  CDR2
  MUTAGEN (1)..(1): Xaa is I, L or V
  MUTAGEN (2)..(2): Xaa is H, T, F, A or S
  MUTAGEN (3)..(3): Xaa is Q, G, S, P, T, I or N
  MUTAGEN (4)..(4): Xaa is G, T, D, A, S or Y
  MUTAGEN (5)..(5): Xaa is G, H, E or N
  MUTAGEN (6)..(6): Xaa is S, E, K, D, G or A
  MUTAGEN (7)..(7): Xaa is T, H, I, K, S or is absent
  MUTAGEN (8)..(8): Xaa is S, T, I, P or is absent
XXXXXXXX

SEQ ID NO: 3 - protein, 25 aa, Artificial Sequence
  CDR3
  MUTAGEN (1)..(1): Xaa is N, S, A, K or H
  MUTAGEN (2)..(2): Xaa is V, I, R, K, A or L
  MUTAGEN (3)..(3): Xaa is V, Y, S, D, L, T or N
  MUTAGEN (4)..(4): Xaa is P, H, L, V, S, K or Y
  MUTAGEN (5)..(5): Xaa is P, Y, S, R, T or A
  MUTAGEN (6)..(6): Xaa is L, P, T, F, A, S or D
  MUTAGEN (7)..(7): Xaa is R, P, F, S, A, I or D
  MUTAGEN (8)..(8): Xaa is V, D, G, A or Y
  MUTAGEN (9)..(9): Xaa is Y, N, T, R, F or is absent
  MUTAGEN (10)..(10): Xaa is P, A, W, E or is absent
  MUTAGEN (11)..(11): Xaa is S, H, L, Y or is absent
  MUTAGEN (12)..(12): Xaa is F, D, N, L or is absent
  MUTAGEN (13)..(13): Xaa is Y, V or is absent
  MUTAGEN (14)..(14): Xaa is I, G or is absent
  MUTAGEN (15)..(15): Xaa is G or is absent
  MUTAGEN (16)..(16): Xaa is Y, A or is absent
  MUTAGEN (17)..(17): Xaa is G or is absent
  MUTAGEN (18)..(18): Xaa is G or is absent
  MUTAGEN (19)..(19): Xaa is G or is absent
  MUTAGEN (20)..(20): Xaa is E or is absent
  MUTAGEN (21)..(21): Xaa is V or is absent
  MUTAGEN (22)..(22): Xaa is R or is absent
  MUTAGEN (23)..(23): Xaa is Y or is absent
  MUTAGEN (24)..(24): Xaa is E or is absent
  MUTAGEN (25)..(25): Xaa is Y or is absent
XXXXXXXXXXXXXXXXXXXXXXXXX

SEQ ID NO: 4 - protein, 8 aa, Artificial Sequence
  CDR1
GSGFTIQA

SEQ ID NO: 5 - protein, 8 aa, Artificial Sequence
  CDR1
GFTFSDYA

SEQ ID NO: 6 - protein, 8 aa, Artificial Sequence
  CDR1
GFTFSDYA

SEQ ID NO: 7 - protein, 8 aa, Artificial Sequence
  CDR1
GFPFETYA

SEQ ID NO: 8 - protein, 8 aa, Artificial Sequence
  CDR1
GFAFSDYT

SEQ ID NO: 9 - protein, 8 aa, Artificial Sequence
  CDR1
GFTFDTYT

SEQ ID NO: 10 - protein, 8 aa, Artificial Sequence
  CDR1
GFSFSDHT

SEQ ID NO: 11 - protein, 8 aa, Artificial Sequence
  CDR1
GLPLLDYA

SEQ ID NO: 12 - protein, 8 aa, Artificial Sequence
  CDR1
GRIDIIFT

SEQ ID NO: 13 - protein, 7 aa, Artificial Sequence
  CDR2
IHQGGST

SEQ ID NO: 14 - protein, 8 aa, Artificial Sequence
  CDR2
ITGTGETS

SEQ ID NO: 15 - protein, 7 aa, Artificial Sequence
  CDR2
ITSGHST

SEQ ID NO: 16 - protein, 8 aa, Artificial Sequence
  CDR2
IFPDGKHT

SEQ ID NO: 17 - protein, 8 aa, Artificial Sequence
  CDR2
ITSAGDII

SEQ ID NO: 18 - protein, 8 aa, Artificial Sequence
  CDR2
LATTGGKP

SEQ ID NO: 19 - protein, 8 aa, Artificial Sequence
  CDR2
ITPAGDII

SEQ ID NO: 20 - protein, 8 aa, Artificial Sequence
  CDR2
ISISEGST

SEQ ID NO: 21 - protein, 6 aa, Artificial Sequence
  CDR2
VTNYNA

SEQ ID NO: 22 - protein, 8 aa, Artificial Sequence
  CDR3
NVVPPLRV

SEQ ID NO: 23 - protein, 9 aa, Artificial Sequence
  CDR3
SIYHPPRDY

SEQ ID NO: 24 - protein, 9 aa, Artificial Sequence
  CDR3
NRSPYTPGN

SEQ ID NO: 25 - protein, 16 aa, Artificial Sequence
  CDR3
AKDLPFFATPSFYIGY

SEQ ID NO: 26 - protein, 13 aa, Artificial Sequence
  CDR3
NALVSASVRASDY

SEQ ID NO: 27 - protein, 13 aa, Artificial Sequence
  CDR3
KATSRSPVNPHNY

SEQ ID NO: 28 - protein, 13 aa, Artificial Sequence
  CDR3
NALVSAAVRASDY

SEQ ID NO: 29 - protein, 25 aa, Artificial Sequence
  CDR3
AADKTDIGFWLLVGGAGGGEVRYEY

SEQ ID NO: 30 - protein, 13 aa, Artificial Sequence
  CDR3
HLNYASDYTEYDY

SEQ ID NO: 31 - protein, 114 aa, Artificial Sequence
  VHH amino acid sequence
EVQLVESGGGLVQPGGSLRLSCTPSGSGFTIQAMTWYRQAPGKQRELVAIIHQGGSTDYSDSVRGRFTISRDNAKTAWYLQMNNLKPEDTAVYYCNVVPPLRVWGQGTQVTVSS

SEQ ID NO: 32 - protein, 116 aa, Artificial Sequence
  VHH amino acid sequence
QVQLVESGGGLVQAGGSLRLSCAASGFTFSDYAVSWYRQAPGKEREFVARITGTGETSRYEDSVKGRFAISRDNVKNTAYLQMNSLKPEDTAVYYCSIYHPPRDYWGQGTQVTVSS

SEQ ID NO: 33 - protein, 115 aa, Artificial Sequence
  VHH amino acid sequence
QVQLVESGGGLVQPGGSLRLSCVASGGVFSSYAMGWYRQVPGKLRELVATITSGHSTTYADIVRGRFTISRDNTKNTVYLQMNRLEPDDTAVYYCNRSPYTPGNWGQGTLVTVSS

SEQ ID NO: 34 - protein, 123 aa, Artificial Sequence
  VHH amino acid sequence
EVQLVESGGGLAQSGGSLRLACEASGFPFETYAMSWARQTPGNEPEWVAGIFPDGKHTAYAHSVKGRFTISRVNANNTVYLQMDSLKPEDTAVYYCAKDLPFFATPSFYIGYWGQGTLVTVSS

SEQ ID NO: 35 - protein, 120 aa, Artificial Sequence
  VHH amino acid sequence
QVQLVESGGGLVQPGGSLRLSCEASGFAFSDYTMRWHRQAAGKELELVAYITSAGDIIKYANSVRGRFTISRDNAKNTLYLQMDSLKPEDTAVYRCNALVSASVRASDYWGQGTLVTVSS

SEQ ID NO: 36 - protein, 120 aa, Artificial Sequence
  VHH amino acid sequence
EVQLVESGGGLVQPGGSLRLSCTASGFTFDTYTTSWERQAPGKEREMVAVLATTGGKPYYVESVKGRFTISRDASETAVTLQMNNLKPEDTAVYYCKATSRSPVNPHNYSGQGTLVTVSS

SEQ ID NO: 37 - protein, 120 aa, Artificial Sequence
  VHH amino acid sequence
EVQLVESGGGLVQPGGSLRLSCEASGFSFSDHTMRWHRQAAGKNLELVAYITPAGDIIKYADSVQGRFTISRDNAKNMLYLQMDSLRPDDTAVYRCNALVSAAVRASDYWGQGTQVTVSS

SEQ ID NO: 38 - protein, 132 aa, Artificial Sequence
  VHH amino acid sequence
EVQVVESGGGLVQSGGSLTLSCTSSGLPLLDYAIGWFRQAPGKEREAVSAISISEGSTYYTDSVRGRFTISRDNNKNKVYLRMDNLKPEDTAVYYCAADKTDIGFWLLVGGAGGGEVRYEYWGQGTQVTVSS

SEQ ID NO: 39 - protein, 118 aa, Artificial Sequence
  VHH amino acid sequence
QVQLVESGGGLVQPGGSLRLSCEASGRIDIIFTMGWYRQTPGNEREFVASVTNYNAKYADSVKGRFTISRENTENTAYLQMNSLKPEDTAIYVCHLNYASDYTEYDYYGQGTQVTVSS

SEQ ID NO: 40 - protein, 116 aa, Artificial Sequence
  amino acid sequence of humanized antibody
EVQLVESGGGLVQPGGSLRLSCAASGFTFSDYAVSWYRQAPGKEREFVSRITGTGETSRYEDSVKGRFTISRDNSKNTAYLQMNSLRAEDTAVYYCSIYHPPRDYWGQGTQVTVSS

SEQ ID NO: 41 - protein, 116 aa, Artificial Sequence
  amino acid sequence of humanized antibody
EVQLVESGGGLVQPGGSLRLSCAASGFTFSDYAVSWYRQAPGKEREFVSRITGTGETSRYEDSVKGRFTISRDNVKNTAYLQMNSLRAEDTAVYYCSIYHPPRDYWGQGTQVTVSS

SEQ ID NO: 42 - protein, 116 aa, Artificial Sequence
  amino acid sequence of humanized antibody
EVQLVESGGGLVQPGGSLRLSCAASGFTFSDYAVSWYRQAPGKEREFVSRITGTGETSRYEDSVKGRFVISRDNSKNTAYLQMNSLRAEDTAVYYCSIYHPPRDYWGQGTQVTVSS

SEQ ID NO: 43 - protein, 116 aa, Artificial Sequence
  amino acid sequence of humanized antibody
EVQLVESGGGLVQPGGSLRLSCAASGFTFSDYAVSWYRQAPGKEREFVARITGTGETSRYEDSVKGRFTISRDNSKNTAYLQMNSLRAEDTAVYYCSIYHPPRDYWGQGTQVTVSS

SEQ ID NO: 44 - protein, 116 aa, Artificial Sequence
  amino acid sequence of humanized antibody
EVQLVESGGGLVQPGGSLRLSCAASGFTFSDYAVSWYRQAPGKEREFVARITGTGETSRYEDSVKGRFTISRDNVKNTAYLQMNSLRAEDTAVYYCSIYHPPRDYWGQGTQVTVSS

SEQ ID NO: 45 - protein, 116 aa, Artificial Sequence
  amino acid sequence of humanized antibody
EVQLVESGGGLVQPGGSLRLSCAASGFTFSDYAVSWYRQAPGKEREFVARITGTGETSRYEDSVKGRFAISRDNSKNTAYLQMNSLRAEDTAVYYCSIYHPPRDYWGQGTQVTVSS

SEQ ID NO: 46 - protein, 116 aa, Artificial Sequence
  amino acid sequence of humanized antibody
EVQLVESGGGLVQPGGSLRLSCAASGFTFSDYAVSWYRQAPGKEREFVARITGTGETSRYEDSVKGRFAISRDNVKNTAYLQMNSLRAEDTAVYYCSIYHPPRDYWGQGTQVTVSS

SEQ ID NO: 47 - protein, 115 aa, Artificial Sequence
  amino acid sequence of humanized antibody
QVQLVESGGGLVQPGGSLRLSCSASGGVFSSYAMGWYRQVPGKLRELVATITSGHSTTYADIVRGRFTISRDNSKNTLYLQMNSLRAEDTAVYYCNRSPYTPGNWGQGTLVTVSS

SEQ ID NO: 48 - protein, 115 aa, Artificial Sequence
  amino acid sequence of humanized antibody
QVQLVESGGGLVQPGGSLRLSCSASGGVFSSYAMGWYRQVPGKLRELVSTITSGHSTTYADIVRGRFTISRDNTKNTLYLQMNSLRAEDTAVYYCNRSPYTPGNWGQGTLVTVSS

SEQ ID NO: 49 - protein, 115 aa, Artificial Sequence
  amino acid sequence of humanized antibody
QVQLVESGGGLVQPGGSLRLSCSASGGVFSSYAMGWYRQVPGKLRELVSTITSGHSTTYADIVRGRFTISRDNSKNTVYLQMNSLRAEDTAVYYCNRSPYTPGNWGQGTLVTVSS

SEQ ID NO: 50 - protein, 115 aa, Artificial Sequence
  amino acid sequence of humanized antibody
QVQLVESGGGLVQPGGSLRLSCSASGGVFSSYAMGWYRQVPGKLRELVATITSGHSTTYADIVRGRFTISRDNTKNTLYLQMNSLRAEDTAVYYCNRSPYTPGNWGQGTLVTVSS

SEQ ID NO: 51 - protein, 115 aa, Artificial Sequence
  amino acid sequence of humanized antibody
QVQLVESGGGLVQPGGSLRLSCSASGGVFSSYAMGWYRQVPGKLRELVATITSGHSTTYADIVRGRFTISRDNSKNTVYLQMNSLRAEDTAVYYCNRSPYTPGNWGQGTLVTVSS

SEQ ID NO: 52 - protein, 115 aa, Artificial Sequence
  amino acid sequence of humanized antibody
QVQLVESGGGLVQPGGSLRLSCSASGGVFSSYAMGWYRQVPGKLRELVATITSGHSTTYADIVRGRFTISRDNTKNTVYLQMNSLRAEDTAVYYCNRSPYTPGNWGQGTLVTVSS

SEQ ID NO: 53 - protein, 115 aa, Artificial Sequence
  amino acid sequence of humanized antibody
QVQLVESGGGLVQPGGSLRLSCSASGGVFSSYAMGWYRQVPGKLRELVSTITSGHSTTYADIVRGRFTISRDNSKNTLYLQMNSLRAEDTAVYYCNRSPYTPGNWGQGTLVTVSS

SEQ ID NO: 54 - protein, 115 aa, Artificial Sequence
  amino acid sequence of humanized antibody
QVQLVESGGGLVQPGGSLRLSCSASGGVFSSYAMGWYRQVPGKLRELVATITSGHSTTYADIVRGRFTISRDNSKNTVYLQMNSLEAEDTAVYYCNRSPYTPGNWGQGTLVTVSS

SEQ ID NO: 55 - protein, 115 aa, Artificial Sequence
  amino acid sequence of humanized antibody
QVQLVESGGGLVQPGGSLRLSCSASGGVFSSYAMGWYRQVPGKLRELVATITSGHSTTYADIVRGRFTISRDNSKNTVYLQMNRLEAEDTAVYYCNRSPYTPGNWGQGTLVTVSS

SEQ ID NO: 56 - protein, 115 aa, Artificial Sequence
  amino acid sequence of humanized antibody
QVQLVESGGGLVQPGGSLRLSCSASGGVFSSYAMGWYRQVPGKLRELVSTITSGHSTTYADIVRGRFTISRDNTKNTVYLQMNRLEAEDTAVYYCNRSPYTPGNWGQGTLVTVSS

SEQ ID NO: 57 - protein, 120 aa, Artificial Sequence
  amino acid sequence of humanized antibody
QVQLVESGGGLVKPGGSLRLSCAASGFAFSDYTMRWHRQAAGKELELVSYITSAGDIIKYANSVRGRFTISRDNAKNTLYLQMNSLRAEDTAVYRCNALVSASVRASDYWGQGTLVTVSS

SEQ ID NO: 58 - protein, 120 aa, Artificial Sequence
  amino acid sequence of humanized antibody
QVQLVESGGGLVKPGGSLRLSCAASGFAFSDYTMRWHRQAAGKELELVAYITSAGDIIKYANSVRGRFTISRDNAKNSLYLQMNSLRAEDTAVYRCNALVSASVRASDYWGQGTLVTVSS

SEQ ID NO: 59 - protein, 120 aa, Artificial Sequence
  amino acid sequence of humanized antibody
QVQLVESGGGLVKPGGSLRLSCAASGFAFSDYTMRWHRQAAGKELELVAYITSAGDIIKYANSVRGRFTISRDNAKNTLYLQMNSLRAEDTAVYRCNALVSASVRASDYWGQGTLVTVSS

SEQ ID NO: 60 - protein, 120 aa, Artificial Sequence
  amino acid sequence of humanized antibody
QVQLVESGGGLVKPGGSLRLSCAASGFAFSDYTMRWHRQAPGKELELVSYITSAGDIIKYANSVRGRFTISRDNAKNSLYLQMNSLRAEDTAVYRCNALVSASVRASDYWGQGTLVTVSS

SEQ ID NO: 61 - protein, 120 aa, Artificial Sequence
  amino acid sequence of humanized antibody
QVQLVESGGGLVKPGGSLRLSCAASGFAFSDYTMRWHRQAPGKELELVAYITSAGDIIKYANSVRGRFTISRDNAKNTLYLQMNSLRAEDTAVYRCNALVSASVRASDYWGQGTLVTVSS

SEQ ID NO: 62 - protein, 120 aa, Artificial Sequence
  amino acid sequence of humanized antibody
QVQLVESGGGLVKPGGSLRLSCAASGFAFSDYTMRWHRQAAGKELELVAYISSAGDIIKYANSVRGRFTISRDNAKNTLYLQMNSLRAEDTAVYRCNALVSASVRASDYWGQGTLVTVSS

SEQ ID NO: 63 - protein, 120 aa, Artificial Sequence
  amino acid sequence of humanized antibody
QVQLVESGGGLVKPGGSLRLSCAASGFAFSDYTMRWHRQAPGKELELVAYITSAGDIIKYANSVRGRFTISRDNAKNSLYLQMNSLRAEDTAVYRCNALVSASVRASDYWGQGTLVTVSS

SEQ ID NO: 64 - protein, 120 aa, Artificial Sequence
  amino acid sequence of humanized antibody
QVQLVESGGGLVKPGGSLRLSCEASGFAFSDYTMRWHRQAAGKELELVAYITSAGDIIKYANSVRGRFTISRDNAKNTLYLQMNSLRAEDTAVYRCNALVSASVRASDYWGQGTLVTVSS

SEQ ID NO: 65 - protein, 120 aa, Artificial Sequence
  amino acid sequence of humanized antibody
EVQLVESGGGLVQPGGSLRLSCAASGFTFDTYTTSWERQAPGKEREMVAVLATTGGKPYYVESVKGRFTISRDNSKNTVYLQMNSLRAEDTAVYYCKATSRSPVNPHNYSGQGTLVTVSS

SEQ ID NO: 66 - protein, 120 aa, Artificial Sequence
  amino acid sequence of humanized antibody
EVQLVESGGGLVQPGGSLRLSCAASGFTFDTYTTSWERQAPGKEREMVAVLATTGGKPYYVESVKGRFTISRDASKNTVYLQMNSLRAEDTAVYYCKATSRSPVNPHNYSGQGTLVTVSS

SEQ ID NO: 67 - protein, 120 aa, Artificial Sequence
  amino acid sequence of humanized antibody
EVQLVESGGGLVQPGGSLRLSCAASGFTFDTYTTSWERQAPGKEREMVAVLATTGGKPYYVESVKGRFTISRDASENTVYLQMNSLRAEDTAVYYCKATSRSPVNPHNYSGQGTLVTVSS

SEQ ID NO: 68 - protein, 120 aa, Artificial Sequence
  amino acid sequence of humanized antibody
EVQLVESGGGLVQPGGSLRLSCAASGFTFDTYTTSWERQAPGKEREMVAVLATTGGKPYYVESVKGRFTISRDASENAVYLQMNSLRAEDTAVYYCKATSRSPVNPHNYSGQGTLVTVSS

SEQ ID NO: 69 - protein, 120 aa, Artificial Sequence
  amino acid sequence of humanized antibody
EVQLVESGGGLVQPGGSLRLSCAASGFTFDTYTTSWERQAPGKEREMVAVLATTGGKPYYVESVKGRFTISRDASENAVYLQMNNLRAEDTAVYYCKATSRSPVNPHNYSGQGTLVTVSS

SEQ ID NO: 70 - protein, 120 aa, Artificial Sequence
  amino acid sequence of humanized antibody
EVQLVESGGGLVQPGGSLRLSCAASGFTFDTYTTSWERQAPGKEREMVAVLATTGGKPYYVESVKGRFTISRDASENAVTLQMNNLRAEDTAVYYCKATSRSPVNPHNYSGQGTLVTVSS

SEQ ID NO: 71 - protein, 120 aa, Artificial Sequence
  amino acid sequence of humanized antibody
EVQLVESGGGLVQPGGSLRLSCAASGFTFDTYTTSWERQAPGKEREMVSVLATTGGKPYYVESVKGRFTISRDASENAVYLQMNSLRAEDTAVYYCKATSRSPVNPHNYSGQGTLVTVSS

SEQ ID NO: 72 - protein, 120 aa, Artificial Sequence
  amino acid sequence of humanized antibody
EVQLVESGGGLVQPGGSLRLSCTASGFTFDTYTTSWERQAPGKEREMVSVLATTGGKPYYVESVKGRFTISRDASENAVTLQMNSLRAEDTAVYYCKATSRSPVNPHNYSGQGTLVTVSS

SEQ ID NO: 73 - protein, 132 aa, Artificial Sequence
  amino acid sequence of humanized antibody
EVQLVESGGGLVQPGGSLRLSCAASGLPLLDYAIGWFRQAPGKEREAVSAISISEGSTYYTDSVRGRFTISRDNSKNTVYLQMNSLRAEDTAVYYCAADKTDIGFWLLVGGAGGGEVRYEYWGQGTQVTVSS

SEQ ID NO: 74 - protein, 132 aa, Artificial Sequence
  amino acid sequence of humanized antibody
EVQLVESGGGLVQPGGSLRLSCAASGLPLLDYAIGWFRQAPGKEREAVSAISISEGSTYYTDSVRGRFTISRDNSKNKLYLQMNSLRAEDTAVYYCAADKTDIGFWLLVGGAGGGEVRYEYWGQGTQVTVSS

SEQ ID NO: 75 - protein, 132 aa, Artificial Sequence
  amino acid sequence of humanized antibody
EVQLVESGGGLVQPGGSLRLSCAASGLPLLDYAIGWFRQAPGKEREAVSAISISEGSTYYTDSVRGRFTISRDNSKNTVYLRMNSLRAEDTAVYYCAADKTDIGFWLLVGGAGGGEVRYEYWGQGTQVTVSS

SEQ ID NO: 76 - protein, 132 aa, Artificial Sequence
  amino acid sequence of humanized antibody
EVQLVESGGGLVQPGGSLRLSCAASGLPLLDYAIGWFRQAPGKEREAVSAISISEGSTYYTDSVRGRFTISRDNNKNTVYLQMNSLRAEDTAVYYCAADKTDIGFWLLVGGAGGGEVRYEYWGQGTQVTVSS

SEQ ID NO: 77 - protein, 132 aa, Artificial Sequence
  amino acid sequence of humanized antibody
EVQLVESGGGLVQPGGSLRLSCAASGLPLLDYAIGWFRQAPGKEREAVSAISISEGSTYYTDSVRGRFTISRDNSKNKVYLQMNSLRAEDTAVYYCAADKTDIGFWLLVGGAGGGEVRYEYWGQGTQVTVSS

SEQ ID NO: 78 - protein, 132 aa, Artificial Sequence
  amino acid sequence of humanized antibody
EVQLVESGGGLVQPGGSLRLSCAASGLPLLDYAIGWFRQAPGKEREAVSAISISEGSTYYTDSVRGRFTISRDNNKNKVYLQMNSLRAEDTAVYYCAADKTDIGFWLLVGGAGGGEVRYEYWGQGTQVTVSS

SEQ ID NO: 79 - protein, 132 aa, Artificial Sequence
  amino acid sequence of humanized antibody
EVQLVESGGGLVQPGGSLRLSCASSGLPLLDYAIGWFRQAPGKEREAVSAISISEGSTYYTDSVRGRFTISRDNNKNKVYLQMNSLRAEDTAVYYCAADKTDIGFWLLVGGAGGGEVRYEYWGQGTQVTVSS

SEQ ID NO: 80 - protein, 132 aa, Artificial Sequence
  amino acid sequence of humanized antibody
EVQLVESGGGLVQPGGSLRLSCSASGLPLLDYAIGWFRQAPGKEREAVSAISISEGSTYYTDSVRGRFTISRDNNKNKVYLQMNSLRAEDTAVYYCAADKTDIGFWLLVGGAGGGEVRYEYWGQGTQVTVSS

SEQ ID NO: 81 - protein, 132 aa, Artificial Sequence
  amino acid sequence of humanized antibody
EVQLVESGGGLVQPGGSLRLSCAASGLPLLDYAIGWFRQAPGKELEAVSAISISEGSTYYTDSVRGRFTISRDNNKNKVYLQMNSLRAEDTAVYYCAADKTDIGFWLLVGGAGGGEVRYEYWGQGTQVTVSS

SEQ ID NO: 82 - protein, 132 aa, Artificial Sequence
  amino acid sequence of humanized antibody
EVQLVESGGGLVQPGGSLRLSCASSGLPLLDYAIGWFRQAPGKEREAVSAISISEGSTYYTDSVRGRFTISRDNSKNKVYLRMNSLRAEDTAVYYCAADKTDIGFWLLVGGAGGGEVRYEYWGQGTQVTVSS

SEQ ID NO: 83 - protein, 229 aa, Artificial Sequence
  CH2 and CH3 of IgG4
ESKYGPPCPPCPAPEFLGGPSVFLFPPKPKDTLMISRTPEVTCVVVDVSQEDPEVQFNWYVDGVEVHNAKTKPREEQFNSTYRVVSVLTVLHQDWLNGKEYKCKVSNKGLPSSIEKTISKAKGQPREPQVYTLPPSQEEMTKNQVSLTCLVKGFYPSDIAVEWESNGQPENNYKTTPPVLDSDGSFFLYSRLTVDKSRWQEGNVFSCSVMHEALHNHYTQKSLSLSLGK

SEQ ID NO: 84 - DNA, 24 bp, Artificial Sequence
  primer
gtcctggctgctcttctacaaggc

SEQ ID NO: 85 - DNA, 23 bp, Artificial Sequence
  primer
ggtacgtgctgttgaactgttcc

SEQ ID NO: 86 - DNA, 29 bp, Artificial Sequence
  primer
gatgtgcagctgcaggagtctggrggagg

SEQ ID NO: 87 - DNA, 35 bp, Artificial Sequence
  primer
ggactagtgcggccgctggagacggtgacctgggt